European Patent Specification EP 3 744 731 B1, published June 18, 2025. Title: LONG-ACTING FGF21 FUSION PROTEINS AND PHARMACEUTICAL COMPOSITION COMPRISING SAME. Applicant: YUHAN CORPORATION. The sequence listing filed with the application follows.

SEQUENCE LISTING (58 sequences)

SEQ ID NO: 1 - protein, 181 aa, human FGF21
HPIPDSSPLLQFGGQVRQRYLYTDDAQQTEAHLEIREDGTVGGAADQSPESLLQLKALKPGVIQILGVKTSRFLCQRPDGALYGSLHFDPEACSFRELLLEDGYNVYQSEAHGLPLHLPGNKSPHRDPAPRGPARFLPLPGLPPALPEPPGILAPQPPDVGSSDPLSMVGPSQGRSPSYAS

SEQ ID NO: 2 - protein, 30 aa, Artificial Sequence
  linker
AKATTAPATTRNTGRGGEEKKKEKEKEEQE

SEQ ID NO: 3 - protein, 17 aa, Artificial Sequence
  linker
AKATTAPATTRNTGRGG

SEQ ID NO: 4 - protein, 15 aa, Artificial Sequence
  linker
GGGGSGGGGSGGGGS

SEQ ID NO: 5 - protein, 16 aa, Artificial Sequence
  linker
GGGGSGGGGSGGGGSA

SEQ ID NO: 6 - protein, 181 aa, Artificial Sequence
  FGF21 variant
HPIPDSSPLLQFGGQVRQRYLYTDDAQQTEAHLEIREDGTVGGAADQSPESLLQLKALKPGVIQILGVKTSRFLCQRPDGALYGSLHFDPEACSFREEIRPDGYNVYQSEAHGLPLHLPGNKSPHRDPAPRGPARFLPLPGLPPALPEPPGILAPQPPDVGSSDPLSMVGPSQGRSPSYAS

SEQ ID NO: 7 - protein, 182 aa, Artificial Sequence
  FGF21 variant
HPIPDSSPLLQFGGQVRQRYLYTDDAQQTEAHLEIREDGTVGGAADQSPESLLQLKALKPGVIQILGVKTSRFLCQRPDGALYGSLHFDPEACSFRELLLEDGYNVYQSEAHGLPLHLPGNKSPHRDPAPRGPARFLPLPGLPPALPEPPGILAPQPPDVGSSDPLSMVTGLEAVRSPSYAS

SEQ ID NO: 8 - protein, 182 aa, Artificial Sequence
  FGF21 variant
HPIPDSSPLLQFGGQVRQRYLYTDDAQQTEAHLEIREDGTVGGAADQSPESLLQLKALKPGVIQILGVKTSRFLCQRPDGALYGSLHFDPEACSFRELLLEDGYNVYQSEAHGLPLHLPGNKSPHRDPAPRGPARFLPLPGLPPALPEPPGILAPQPPDVGSSDPLSMVTGLEANRSPSYAS

SEQ ID NO: 9 - protein, 181 aa, Artificial Sequence
  FGF21 variant
HPIPDSSPLLQFGGQVRQRYLYTDDAQQTEAHLEIREDGTVGGAADQSPESLLQLKALKPGVIQILGVKTSRFLCQRPDGALYGSLHFDPEACSFRELLLEDGYNVYQSEAHGLPLHLPGNKSPHRDPAPRGPARFLPLPGLPPALPEPPGILAPQPPDVGSSDPLSMVNPSQGRSPSYAS

SEQ ID NO: 10 - protein, 181 aa, Artificial Sequence
  FGF21 variant
HPIPDSSPLLQFGGQVRQRYLYTDDAQQTEAHLEIREDGTVGGAADQSPESLLQLKALKPGVIQILGVKTSRFLCQRPDGALYGSLHFDPEACSFRELLLEDGYNVYQSEAHGLPLHLPGNKSPHRDPAPRGPARFLPLPGLPPALPEPPGILAPQPPDVGSSDPLSMVGPSQNRSPSYAS

SEQ ID NO: 11 - protein, 182 aa, Artificial Sequence
  FGF21 variant
HPIPDSSPLLQFGGQVRQRYLYTDDAQQTEAHLEIREDGTVGGAADQSPESLLQLKALKPGVIQILGVKTSRFLCQRPDGALYGSLHFDPEACSFREEIRPDGYNVYQSEAHGLPLHLPGNKSPHRDPAPRGPARFLPLPGLPPALPEPPGILAPQPPDVGSSDPLSMVTGLEAVRSPSYAS

SEQ ID NO: 12 - protein, 182 aa, Artificial Sequence
  FGF21 variant
HPIPDSSPLLQFGGQVRQRYLYTDDAQQTEAHLEIREDGTVGGAADQSPESLLQLKALKPGVIQILGVKTSRFLCQRPDGALYGSLHFDPEACSFREEIRPDGYNVYQSEAHGLPLHLPGNKSPHRDPAPRGPARFLPLPGLPPALPEPPGILAPQPPDVGSSDPLSMVTGLEANRSPSYAS

SEQ ID NO: 13 - protein, 181 aa, Artificial Sequence
  FGF21 variant
HPIPDSSPLLQFGGQVRQRYLYTDDAQQTEAHLEIREDGTVGGAADQSPESLLQLKALKPGVIQILGVKTSRFLCQRPDGALYGSLHFDPEACSFREEIRPDGYNVYQSEAHGLPLHLPGNKSPHRDPAPRGPARFLPLPGLPPALPEPPGILAPQPPDVGSSDPLSMVNPSQGRSPSYAS

SEQ ID NO: 14 - protein, 181 aa, Artificial Sequence
  FGF21 variant
HPIPDSSPLLQFGGQVRQRYLYTDDAQQTEAHLEIREDGTVGGAADQSPESLLQLKALKPGVIQILGVKTSRFLCQRPDGALYGSLHFDPEACSFREEIRPDGYNVYQSEAHGLPLHLPGNKSPHRDPAPRGPARFLPLPGLPPALPEPPGILAPQPPDVGSSDPLSMVGPSQNRSPSYAS

SEQ ID NO: 15 - protein, 181 aa, Artificial Sequence
  FGF21 variant
HPIPDSSPLLQFGGQVRQRYLYTDDAQQTEAHLEIREDGTVGGAADQSPESLLQLKALKPGVIQILGVKTSRFLCQRPDGALYGSLHFDPEACSFREEIRPDGYNVYQSEAHGLPLHLPGNKSPHRDPAPRGPARFLPLPGLPPALPEPPGILAPQPPDVGSSDPLSMVGPSQGRSPSYES

SEQ ID NO: 16 - protein, 182 aa, Artificial Sequence
  FGF21 variant
HPIPDSSPLLQFGGQVRQRYLYTDDAQQTEAHLEIREDGTVGGAADQSPESLLQLKALKPGVIQILGVKTSRFLCQRPDGALYGSLHFDPEACSFRELLLEDGYNVYQSEAHGLPLHLPGNKSPHRDPAPRGPARFLPLPGLPPALPEPPGILAPQPPDVGSSDPLSMVTGLEAVRSPSYES

SEQ ID NO: 17 - protein, 182 aa, Artificial Sequence
  FGF21 variant
HPIPDSSPLLQFGGQVRQRYLYTDDAQQTEAHLEIREDGTVGGAADQSPESLLQLKALKPGVIQILGVKTSRFLCQRPDGALYGSLHFDPEACSFRELLLEDGYNVYQSEAHGLPLHLPGNKSPHRDPAPRGPARFLPLPGLPPALPEPPGILAPQPPDVGSSDPLSMVTGLEANRSPSYES

SEQ ID NO: 18 - protein, 181 aa, Artificial Sequence
  FGF21 variant
HPIPDSSPLLQFGGQVRQRYLYTDDAQQTEAHLEIREDGTVGGAADQSPESLLQLKALKPGVIQILGVKTSRFLCQRPDGALYGSLHFDPEACSFRELLLEDGYNVYQSEAHGLPLHLPGNKSPHRDPAPRGPARFLPLPGLPPALPEPPGILAPQPPDVGSSDPLSMVNPSQGRSPSYES

SEQ ID NO: 19 - protein, 181 aa, Artificial Sequence
  FGF21 variant
HPIPDSSPLLQFGGQVRQRYLYTDDAQQTEAHLEIREDGTVGGAADQSPESLLQLKALKPGVIQILGVKTSRFLCQRPDGALYGSLHFDPEACSFRELLLEDGYNVYQSEAHGLPLHLPGNKSPHRDPAPRGPARFLPLPGLPPALPEPPGILAPQPPDVGSSDPLSMVGPSQNRSPSYES

SEQ ID NO: 20 - protein, 182 aa, Artificial Sequence
  FGF21 variant
HPIPDSSPLLQFGGQVRQRYLYTDDAQQTEAHLEIREDGTVGGAADQSPESLLQLKALKPGVIQILGVKTSRFLCQRPDGALYGSLHFDPEACSFREEIRPDGYNVYQSEAHGLPLHLPGNKSPHRDPAPRGPARFLPLPGLPPALPEPPGILAPQPPDVGSSDPLSMVTGLEAVRSPSYES

SEQ ID NO: 21 - protein, 182 aa, Artificial Sequence
  FGF21 variant
HPIPDSSPLLQFGGQVRQRYLYTDDAQQTEAHLEIREDGTVGGAADQSPESLLQLKALKPGVIQILGVKTSRFLCQRPDGALYGSLHFDPEACSFREEIRPDGYNVYQSEAHGLPLHLPGNKSPHRDPAPRGPARFLPLPGLPPALPEPPGILAPQPPDVGSSDPLSMVTGLEANRSPSYES

SEQ ID NO: 22 - protein, 181 aa, Artificial Sequence
  FGF21 variant
HPIPDSSPLLQFGGQVRQRYLYTDDAQQTEAHLEIREDGTVGGAADQSPESLLQLKALKPGVIQILGVKTSRFLCQRPDGALYGSLHFDPEACSFREEIRPDGYNVYQSEAHGLPLHLPGNKSPHRDPAPRGPARFLPLPGLPPALPEPPGILAPQPPDVGSSDPLSMVNPSQGRSPSYES

SEQ ID NO: 23 - protein, 181 aa, Artificial Sequence
  FGF21 variant
HPIPDSSPLLQFGGQVRQRYLYTDDAQQTEAHLEIREDGTVGGAADQSPESLLQLKALKPGVIQILGVKTSRFLCQRPDGALYGSLHFDPEACSFREEIRPDGYNVYQSEAHGLPLHLPGNKSPHRDPAPRGPARFLPLPGLPPALPEPPGILAPQPPDVGSSDPLSMVGPSQNRSPSYES

SEQ ID NO: 24 - protein, 229 aa, Artificial Sequence
  Human IgG4 Fc
ESKYGPPCPSCPAPEFLGGPSVFLFPPKPKDTLMISRTPEVTCVVVDVSQEDPEVQFNWYVDGVEVHNAKTKPREEQFNSTYRVVSVLTVLHQDWLNGKEYKCKVSNKGLPSSIEKTISKAKGQPREPQVYTLPPSQEEMTKNQVSLTCLVKGFYPSDIAVEWESNGQPENNYKTTPPVLDSDGSFFLYSRLTVDKSRWQEGNVFSCSVMHEALHNHYTQKSLSLSLGK

SEQ ID NO: 25 - protein, 228 aa, Artificial Sequence
  Human IgG4 Fc variant
ESKYGPPCPPCPAPEAAGGPSVFLFPPKPKDTLMISRTPEVTCVVVDVSQEDPEVQFNWYVDGVEVHNAKTKPREEQFNSTYRVVSVLTVLHQDWLNGKEYKCKVSNKGLPSSIEKTISKAKGQPREPQVYTLPPSQEEMTKNQVSLTCLVKGFYPSDIAVEWESNGQPENNYKTTPPVLDSDGSFFLYSRLTVDKSRWQEGNVFSCSVMHEALHNHYTQKSLSLSLG

SEQ ID NO: 26 - protein, 223 aa, Artificial Sequence
  Hybrid Fc variant
ETKTPECPSHTQPLGVFLFPPKPKDTLMISRTPEVTCVVVDVSQEDPEVQFNWYVDGVEVHNAKTKPREEQFNSTYRVVSVLTVLHQDWLNGKEYKCKVSNKGLPSSIEKTISKAKGQPREPQVYTLPPSQEEMTKNQVSLTCLVKGFYPSDIAVEWESNGQPENNYKTTPPVLDSDGSFFLYSRLTVDKSRWQEGNVFSCSVMHEALHNHYTQKSLSLSLGK

SEQ ID NO: 27 - protein, 435 aa, Artificial Sequence
  modified FGF21 variant connected to hybrid Fc
ETKTPECPSHTQPLGVFLFPPKPKDTLMISRTPEVTCVVVDVSQEDPEVQFNWYVDGVEVHNAKTKPREEQFNSTYRVVSVLTVLHQDWLNGKEYKCKVSNKGLPSSIEKTISKAKGQPREPQVYTLPPSQEEMTKNQVSLTCLVKGFYPSDIAVEWESNGQPENNYKTTPPVLDSDGSFFLYSRLTVDKSRWQEGNVFSCSVMHEALHNHYTQKSLSLSLGKAKATTAPATTRNTGRGGEEKKKEKEKEEQEHPIPDSSPLLQFGGQVRQRYLYTDDAQQTEAHLEIREDGTVGGAADQSPESLLQLKALKPGVIQILGVKTSRFLCQRPDGALYGSLHFDPEACSFREEIRPDGYNVYQSEAHGLPLHLPGNKSPHRDPAPRGPARFLPLPGLPPALPEPPGILAPQPPDVGSSDPLSMVTGLEAVRSPSYAS

SEQ ID NO: 28 - protein, 422 aa, Artificial Sequence
  modified FGF21 variant connected to hybrid Fc
ETKTPECPSHTQPLGVFLFPPKPKDTLMISRTPEVTCVVVDVSQEDPEVQFNWYVDGVEVHNAKTKPREEQFNSTYRVVSVLTVLHQDWLNGKEYKCKVSNKGLPSSIEKTISKAKGQPREPQVYTLPPSQEEMTKNQVSLTCLVKGFYPSDIAVEWESNGQPENNYKTTPPVLDSDGSFFLYSRLTVDKSRWQEGNVFSCSVMHEALHNHYTQKSLSLSLGKAKATTAPATTRNTGRGGHPIPDSSPLLQFGGQVRQRYLYTDDAQQTEAHLEIREDGTVGGAADQSPESLLQLKALKPGVIQILGVKTSRFLCQRPDGALYGSLHFDPEACSFRELLLEDGYNVYQSEAHGLPLHLPGNKSPHRDPAPRGPARFLPLPGLPPALPEPPGILAPQPPDVGSSDPLSMVTGLEAVRSPSYAS

SEQ ID NO: 29 - protein, 420 aa, Artificial Sequence
  modified FGF21 variant connected to hybrid Fc
ETKTPECPSHTQPLGVFLFPPKPKDTLMISRTPEVTCVVVDVSQEDPEVQFNWYVDGVEVHNAKTKPREEQFNSTYRVVSVLTVLHQDWLNGKEYKCKVSNKGLPSSIEKTISKAKGQPREPQVYTLPPSQEEMTKNQVSLTCLVKGFYPSDIAVEWESNGQPENNYKTTPPVLDSDGSFFLYSRLTVDKSRWQEGNVFSCSVMHEALHNHYTQKSLSLSLGKGGGGSGGGGSGGGGSHPIPDSSPLLQFGGQVRQRYLYTDDAQQTEAHLEIREDGTVGGAADQSPESLLQLKALKPGVIQILGVKTSRFLCQRPDGALYGSLHFDPEACSFRELLLEDGYNVYQSEAHGLPLHLPGNKSPHRDPAPRGPARFLPLPGLPPALPEPPGILAPQPPDVGSSDPLSMVTGLEAVRSPSYAS

SEQ ID NO: 30 - protein, 420 aa, Artificial Sequence
  modified FGF21 variant connected to hybrid Fc
ETKTPECPSHTQPLGVFLFPPKPKDTLMISRTPEVTCVVVDVSQEDPEVQFNWYVDGVEVHNAKTKPREEQFNSTYRVVSVLTVLHQDWLNGKEYKCKVSNKGLPSSIEKTISKAKGQPREPQVYTLPPSQEEMTKNQVSLTCLVKGFYPSDIAVEWESNGQPENNYKTTPPVLDSDGSFFLYSRLTVDKSRWQEGNVFSCSVMHEALHNHYTQKSLSLSLGKGGGGSGGGGSGGGGSHPIPDSSPLLQFGGQVRQRYLYTDDAQQTEAHLEIREDGTVGGAADQSPESLLQLKALKPGVIQILGVKTSRFLCQRPDGALYGSLHFDPEACSFRELLLEDGYNVYQSEAHGLPLHLPGNKSPHRDPAPRGPARFLPLPGLPPALPEPPGILAPQPPDVGSSDPLSMVTGLEANRSPSYAS

SEQ ID NO: 31 - protein, 419 aa, Artificial Sequence
  modified FGF21 variant connected to hybrid Fc
ETKTPECPSHTQPLGVFLFPPKPKDTLMISRTPEVTCVVVDVSQEDPEVQFNWYVDGVEVHNAKTKPREEQFNSTYRVVSVLTVLHQDWLNGKEYKCKVSNKGLPSSIEKTISKAKGQPREPQVYTLPPSQEEMTKNQVSLTCLVKGFYPSDIAVEWESNGQPENNYKTTPPVLDSDGSFFLYSRLTVDKSRWQEGNVFSCSVMHEALHNHYTQKSLSLSLGKGGGGSGGGGSGGGGSHPIPDSSPLLQFGGQVRQRYLYTDDAQQTEAHLEIREDGTVGGAADQSPESLLQLKALKPGVIQILGVKTSRFLCQRPDGALYGSLHFDPEACSFRELLLEDGYNVYQSEAHGLPLHLPGNKSPHRDPAPRGPARFLPLPGLPPALPEPPGILAPQPPDVGSSDPLSMVNPSQGRSPSYAS

SEQ ID NO: 32 - protein, 419 aa, Artificial Sequence; identical to SEQ ID NO: 31
  modified FGF21 variant connected to hybrid Fc

SEQ ID NO: 33 - protein, 419 aa, Artificial Sequence
  modified FGF21 variant connected to hybrid Fc
ETKTPECPSHTQPLGVFLFPPKPKDTLMISRTPEVTCVVVDVSQEDPEVQFNWYVDGVEVHNAKTKPREEQFNSTYRVVSVLTVLHQDWLNGKEYKCKVSNKGLPSSIEKTISKAKGQPREPQVYTLPPSQEEMTKNQVSLTCLVKGFYPSDIAVEWESNGQPENNYKTTPPVLDSDGSFFLYSRLTVDKSRWQEGNVFSCSVMHEALHNHYTQKSLSLSLGKGGGGSGGGGSGGGGSHPIPDSSPLLQFGGQVRQRYLYTDDAQQTEAHLEIREDGTVGGAADQSPESLLQLKALKPGVIQILGVKTSRFLCQRPDGALYGSLHFDPEACSFRELLLEDGYNVYQSEAHGLPLHLPGNKSPHRDPAPRGPARFLPLPGLPPALPEPPGILAPQPPDVGSSDPLSMVGPSQNRSPSYAS

SEQ ID NO: 34 - protein, 419 aa, Artificial Sequence
  modified FGF21 variant connected to hybrid Fc
ETKTPECPSHTQPLGVFLFPPKPKDTLMISRTPEVTCVVVDVSQEDPEVQFNWYVDGVEVHNAKTKPREEQFNSTYRVVSVLTVLHQDWLNGKEYKCKVSNKGLPSSIEKTISKAKGQPREPQVYTLPPSQEEMTKNQVSLTCLVKGFYPSDIAVEWESNGQPENNYKTTPPVLDSDGSFFLYSRLTVDKSRWQEGNVFSCSVMHEALHNHYTQKSLSLSLGKGGGGSGGGGSGGGGSHPIPDSSPLLQFGGQVRQRYLYTDDAQQTEAHLEIREDGTVGGAADQSPESLLQLKALKPGVIQILGVKTSRFLCQRPDGALYGSLHFDPEACSFRELLLEDGYNVYQSEAHGLPLHLPGNKSPHRDPAPRGPARFLPLPGLPPALPEPPGILAPQPPDVGSSDPLSMVGPSQGRSPSYAS

SEQ ID NO: 35 - protein, 420 aa, Artificial Sequence
  modified FGF21 variant connected to hybrid Fc
ETKTPECPSHTQPLGVFLFPPKPKDTLMISRTPEVTCVVVDVSQEDPEVQFNWYVDGVEVHNAKTKPREEQFNSTYRVVSVLTVLHQDWLNGKEYKCKVSNKGLPSSIEKTISKAKGQPREPQVYTLPPSQEEMTKNQVSLTCLVKGFYPSDIAVEWESNGQPENNYKTTPPVLDSDGSFFLYSRLTVDKSRWQEGNVFSCSVMHEALHNHYTQKSLSLSLGKGGGGSGGGGSGGGGSHPIPDSSPLLQFGGQVRQRYLYTDDAQQTEAHLEIREDGTVGGAADQSPESLLQLKALKPGVIQILGVKTSRFLCQRPDGALYGSLHFDPEACSFREEIRPDGYNVYQSEAHGLPLHLPGNKSPHRDPAPRGPARFLPLPGLPPALPEPPGILAPQPPDVGSSDPLSMVTGLEAVRSPSYAS

SEQ ID NO: 36 - protein, 420 aa, Artificial Sequence
  modified FGF21 variant connected to hybrid Fc
ETKTPECPSHTQPLGVFLFPPKPKDTLMISRTPEVTCVVVDVSQEDPEVQFNWYVDGVEVHNAKTKPREEQFNSTYRVVSVLTVLHQDWLNGKEYKCKVSNKGLPSSIEKTISKAKGQPREPQVYTLPPSQEEMTKNQVSLTCLVKGFYPSDIAVEWESNGQPENNYKTTPPVLDSDGSFFLYSRLTVDKSRWQEGNVFSCSVMHEALHNHYTQKSLSLSLGKGGGGSGGGGSGGGGSHPIPDSSPLLQFGGQVRQRYLYTDDAQQTEAHLEIREDGTVGGAADQSPESLLQLKALKPGVIQILGVKTSRFLCQRPDGALYGSLHFDPEACSFREEIRPDGYNVYQSEAHGLPLHLPGNKSPHRDPAPRGPARFLPLPGLPPALPEPPGILAPQPPDVGSSDPLSMVTGLEAVRSPSYES

SEQ ID NO: 37 - protein, 420 aa, Artificial Sequence
  modified FGF21 variant connected to hybrid Fc
ETKTPECPSHTQPLGVFLFPPKPKDTLMISRTPEVTCVVVDVSQEDPEVQFNWYVDGVEVHNAKTKPREEQFNSTYRVVSVLTVLHQDWLNGKEYKCKVSNKGLPSSIEKTISKAKGQPREPQVYTLPPSQEEMTKNQVSLTCLVKGFYPSDIAVEWESNGQPENNYKTTPPVLDSDGSFFLYSRLTVDKSRWQEGNVFSCSVMHEALHNHYTQKSLSLSLGKGGGGSGGGGSGGGGSHPIPDSSPLLQFGGQVRQRYLYTDDAQQTEAHLEIREDGTVGGAADQSPESLLQLKALKPGVIQILGVKTSRFLCQRPDGALYGSLHFDPEACSFREEIRPDGYNVYQSEAHGLPLHLPGNKSPHRDPAPRGPARFLPLPGLPPALPEPPGILAPQPPDVGSSDPLSMVTGLEANRSPSYES

SEQ ID NO: 38 - protein, 419 aa, Artificial Sequence
  modified FGF21 variant connected to hybrid Fc
ETKTPECPSHTQPLGVFLFPPKPKDTLMISRTPEVTCVVVDVSQEDPEVQFNWYVDGVEVHNAKTKPREEQFNSTYRVVSVLTVLHQDWLNGKEYKCKVSNKGLPSSIEKTISKAKGQPREPQVYTLPPSQEEMTKNQVSLTCLVKGFYPSDIAVEWESNGQPENNYKTTPPVLDSDGSFFLYSRLTVDKSRWQEGNVFSCSVMHEALHNHYTQKSLSLSLGKGGGGSGGGGSGGGGSHPIPDSSPLLQFGGQVRQRYLYTDDAQQTEAHLEIREDGTVGGAADQSPESLLQLKALKPGVIQILGVKTSRFLCQRPDGALYGSLHFDPEACSFREEIRPDGYNVYQSEAHGLPLHLPGNKSPHRDPAPRGPARFLPLPGLPPALPEPPGILAPQPPDVGSSDPLSMVNPSQGRSPSYAS

SEQ ID NO: 39 - protein, 419 aa, Artificial Sequence
  modified FGF21 variant connected to hybrid Fc
ETKTPECPSHTQPLGVFLFPPKPKDTLMISRTPEVTCVVVDVSQEDPEVQFNWYVDGVEVHNAKTKPREEQFNSTYRVVSVLTVLHQDWLNGKEYKCKVSNKGLPSSIEKTISKAKGQPREPQVYTLPPSQEEMTKNQVSLTCLVKGFYPSDIAVEWESNGQPENNYKTTPPVLDSDGSFFLYSRLTVDKSRWQEGNVFSCSVMHEALHNHYTQKSLSLSLGKGGGGSGGGGSGGGGSHPIPDSSPLLQFGGQVRQRYLYTDDAQQTEAHLEIREDGTVGGAADQSPESLLQLKALKPGVIQILGVKTSRFLCQRPDGALYGSLHFDPEACSFREEIRPDGYNVYQSEAHGLPLHLPGNKSPHRDPAPRGPARFLPLPGLPPALPEPPGILAPQPPDVGSSDPLSMVNPSQGRSPSYES

SEQ ID NO: 40 - protein, 423 aa, Artificial Sequence
  RGE(Amgen)
DKTHTCPPCPAPELLGGPSVFLFPPKPKDTLMISRTPEVTCVVVDVSHEDPEVKFNWYVDGVEVHNAKTKPREEQYNSTYRVVSVLTVLHQDWLNGKEYKCKVSNKALPAPIEKTISKAKGQPREPQVYTLPPSRDELTKNQVSLTCLVKGFYPSDIAVEWESNGQPENNYKTTPPVLDSDGSFFLYSKLTVDKSRWQQGNVFSCSVMHEALHNHYTQKSLSLSPGKGGGGSGGGGSGGGGSHPIPDSSPLLQFGGQVRQRYLYTDDAQQTEAHLEIREDGTVGGAADQSPESLLQLKALKPGVIQILGVKTSRFLCQRPDGALYGSLHFDPEACSFRERLLEDGYNVYQSEAHGLPLHLPGNKSPHRDPAPRGPARFLPLPGLPPALPEPPGILAPQPPDVGSSDPLSMVGGSQGRSPSYES

SEQ ID NO: 41 - protein, 424 aa, Artificial Sequence
  FGF21 connected to Fc(lilly)
ESKYGPPCPPCPAPEAAGGPSVFLFPPKPKDTLMISRTPEVTCVVVDVSQEDPEVQFNWYVDGVEVHNAKTKPREEQFNSTYRVVSVLTVLHQDWLNGKEYKCKVSNKGLPSSIEKTISKAKGQPREPQVYTLPPSQEEMTKNQVSLTCLVKGFYPSDIAVEWESNGQPENNYKTTPPVLDSDGSFFLYSRLTVDKSRWQEGNVFSCSVMHEALHNHYTQKSLSLSLGGGGGSGGGGSGGGGSAHPIPDSSPLLQFGGQVRQRYLYTDDAQQTECHLEIREDGTVGCAADQSPESLLQLKALKPGVIQILGVKTSRFLCQRPDGALYGSLHFDPEACSFREDLKEDGYNVYQSEAHGLPLHLPGDKSPHRKPAPRGPARFLPLPGLPPALPEPPGILAPQPPDVGSSDPLRLVEPSQLRSPSFE

SEQ ID NO: 42 - protein, 4 aa, Artificial Sequence
  FGF21 variant
EIRP

SEQ ID NO: 43 - protein, 6 aa, Artificial Sequence
  FGF21 variant
TGLEAV

SEQ ID NO: 44 - protein, 6 aa, Artificial Sequence
  FGF21 variant
TGLEAN

SEQ ID NO: 45 - DNA, 1305 bp, Artificial Sequence
  nucleic acid molecule coding for DFD1
gagaccaagacacctgaatgtccaagtcacactcagcctctgggagtgtttctcttcccacctaagcccaaggatacccttatgatttctaggacacctgaggtgacctgcgtcgttgtggacgtgagtcaagaggacccagaggtccagtttaactggtatgttgacggcgtggaagtgcataatgcaaaaactaaaccccgcgaggaacaattcaattcaacctaccgggtcgtttctgtgttgacagtgctgcatcaagattggctgaacgggaaggagtataagtgtaaagtcagtaataagggactcccctctagtatcgaaaaaactatttcaaaggccaaaggccagcctagagagccacaggtttacacccttcctccatcccaagaggagatgacaaagaaccaggtgtctctgacttgtctcgtgaaggggttctaccctagtgacatcgctgtcgaatgggagtcaaacggacagccagagaataattataagacaactcctcccgttctggattctgacggcagcttctttctgtactctaggcttactgtggacaaaagtcgctggcaagaagggaacgtcttttcatgttctgttatgcacgaggccttgcacaatcattatacacagaagtctctgagtctctcactgggcaaagccaaggctaccacagcacccgccactacccggaacaccggtagagggggagaggaaaagaagaaagagaaggaaaaagaggaacaggagcatcccatccctgactccagtcctctcctgcaattcgggggccaagtccggcagcggtacctctacacagatgatgctcagcagacagaagcccacctggagatcagggaggatgggaccgtggggggcgctgctgaccagagccccgaaagtctcctgcagctgaaagccttgaagcctggagttattcaaatcttgggagtcaagactagtaggttcctgtgccagcggccagatggggccctgtatggatctctccattttgaccctgaggcctgcagcttccgggaggagatcagacccgacggatacaatgtttaccagtccgaagcccacggcctccctctgcatctgcccgggaacaagtctcctcaccgggaccctgcccccagaggacctgctcgcttcctgccactcccaggcctgccccccgcattgcctgagccacccggaatcctggccccccagccccctgatgtgggatcctctgaccctctgagcatggtgacaggcctggaggccgtgagaagccccagctacgcttcc

SEQ ID NO: 46 - DNA, 1266 bp, Artificial Sequence
  nucleic acid molecule coding for DFD3
gagaccaagacacctgaatgtccaagtcacactcagcctctgggagtgtttctcttcccacctaagcccaaggatacccttatgatttctaggacacctgaggtgacctgcgtcgttgtggacgtgagtcaagaggacccagaggtccagtttaactggtatgttgacggcgtggaagtgcataatgcaaaaactaaaccccgcgaggaacaattcaattcaacctaccgggtcgtttctgtgttgacagtgctgcatcaagattggctgaacgggaaggagtataagtgtaaagtcagtaataagggactcccctctagtatcgaaaaaactatttcaaaggccaaaggccagcctagagagccacaggtgtacacccttcctccatcccaagaggagatgacaaagaaccaggtgtctctgacttgtctcgtgaaggggttctaccctagtgacatcgctgtcgaatgggagtcaaacggacagccagagaataattataagacaactcctcccgttctggattctgacggcagcttctttctgtactctaggcttactgtggacaaaagtcgctggcaagaagggaacgtcttttcatgttctgttatgcacgaggccttgcacaatcattatacacagaagtctctgagtctctcactgggcaaagccaaggctaccacagcacccgccactaccagaaacacaggcagggggggacatcccatccctgactccagtcctctcctgcaattcgggggccaagtccggcagcggtacctctacacagatgatgctcagcagacagaagcccacctggagatcagggaggatgggaccgtggggggcgctgctgaccagagccccgaaagtctcctgcagctgaaagccttgaagcctggagttattcaaatcttgggagtcaagactagtaggttcctgtgccagcggccagatggggccctgtatggatctctccattttgaccctgaggcctgcagcttccgggagctgcttcttgaggacggatacaatgtttaccagtccgaagcccacggcctccctctgcatctgcccgggaacaagtctcctcaccgggaccctgcccccagaggacctgctcgcttcctgccactcccaggcctgccccccgcattgcctgagccacccggaatcctggccccccagccccctgatgtgggatcctctgaccctctgagcatggtgacaggcctggaggccgtgagaagccccagctacgcttcc

SEQ ID NO: 47 - DNA, 1260 bp, Artificial Sequence
  nucleic acid molecule coding for DFD4
gagaccaagacacctgaatgtccaagtcacactcagcctctgggagtgtttctcttcccacctaagcccaaggatacccttatgatttctaggacacctgaggtgacctgcgtcgttgtggacgtgagtcaagaggacccagaggtccagtttaactggtatgttgacggcgtggaagtgcataatgcaaaaactaaaccccgcgaggaacaattcaattcaacctaccgggtcgtttctgtgttgacagtgctgcatcaagattggctgaacgggaaggagtataagtgtaaagtcagtaataagggactcccctctagtatcgaaaaaactatttcaaaggccaaaggccagcctagagagccacaggtgtacacccttcctccatcccaagaggagatgacaaagaaccaggtgtctctgacttgtctcgtgaaggggttctaccctagtgacatcgctgtcgaatgggagtcaaacggacagccagagaataattataagacaactcctcccgttctggattctgacggcagcttctttctgtactctaggcttactgtggacaaaagtcgctggcaagaagggaacgtcttttcatgttctgttatgcacgaggccttgcacaatcattatacacagaagtctctgagtctctcactgggcaaaggcgggggaggcagcgggggaggcgggtccggaggcgggggatctcatcccatccctgactccagtcctctcctgcaattcgggggccaagtccggcagcggtacctctacacagatgatgctcagcagacagaagcccacctggagatcagggaggatgggaccgtggggggcgctgctgaccagagccccgaaagtctcctgcagctgaaagccttgaagcctggagttattcaaatcttgggagtcaagactagtaggttcctgtgccagcggccagatggggccctgtatggatctctccattttgaccctgaggcctgcagcttccgggagctgcttcttgaggacggatacaatgtttaccagtccgaagcccacggcctccctctgcatctgcccgggaacaagtctcctcaccgggaccctgcccccagaggacctgctcgcttcctgccactcccaggcctgccccccgcattgcctgagccacccggaatcctggccccccagccccctgatgtgggatcctctgaccctctgagcatggtgacaggcctggaggccgtgagaagccccagctacgcttcc

SEQ ID NO: 48 - DNA, 1260 bp, Artificial Sequence
  nucleic acid molecule coding for DFD5
gagaccaagacacctgaatgtccaagtcacactcagcctctgggagtgtttctcttcccacctaagcccaaggatacccttatgatttctaggacacctgaggtgacctgcgtcgttgtggacgtgagtcaagaggacccagaggtccagtttaactggtatgttgacggcgtggaagtgcataatgcaaaaactaaaccccgcgaggaacaattcaattcaacctaccgggtcgtttctgtgttgacagtgctgcatcaagattggctgaacgggaaggagtataagtgtaaagtcagtaataagggactcccctctagtatcgaaaaaactatttcaaaggccaaaggccagcctagagagccacaggtgtacacccttcctccatcccaagaggagatgacaaagaaccaggtgtctctgacttgtctcgtgaaggggttctaccctagtgacatcgctgtcgaatgggagtcaaacggacagccagagaataattataagacaactcctcccgttctggattctgacggcagcttctttctgtactctaggcttactgtggacaaaagtcgctggcaagaagggaacgtcttttcatgttctgttatgcacgaggccttgcacaatcattatacacagaagtctctgagtctctcactgggcaaaggcgggggaggcagcgggggaggcgggtccggaggcgggggatctcatcccatccctgactccagtcctctcctgcaattcgggggccaagtccggcagcggtacctctacacagatgatgctcagcagacagaagcccacctggagatcagggaggatgggaccgtggggggcgctgctgaccagagccccgaaagtctcctgcagctgaaagccttgaagcctggagttattcaaatcttgggagtcaagactagtaggttcctgtgccagcggccagatggggccctgtatggatctctccattttgaccctgaggcctgcagcttccgggagctgcttcttgaggacggatacaatgtttaccagtccgaagcccacggcctccctctgcatctgcccgggaacaagtctcctcaccgggaccctgcccccagaggacctgctcgcttcctgccactcccaggcctgccccccgcattgcctgagccacccggaatcctggccccccagccccctgatgtgggatcctctgaccctctgagcatggtgacaggcctggaggccaacagaagccccagctacgcttcc

SEQ ID NO: 49 - DNA, 1257 bp, Artificial Sequence
  nucleic acid molecule coding for DFD6
gagaccaagacacctgaatgtccaagtcacactcagcctctgggagtgtttctcttcccacctaagcccaaggatacccttatgatttctaggacacctgaggtgacctgcgtcgttgtggacgtgagtcaagaggacccagaggtccagtttaactggtatgttgacggcgtggaagtgcataatgcaaaaactaaaccccgcgaggaacaattcaattcaacctaccgggtcgtttctgtgttgacagtgctgcatcaagattggctgaacgggaaggagtataagtgtaaagtcagtaataagggactcccctctagtatcgaaaaaactatttcaaaggccaaaggccagcctagagagccacaggtgtacacccttcctccatcccaagaggagatgacaaagaaccaggtgtctctgacttgtctcgtgaaggggttctaccctagtgacatcgctgtcgaatgggagtcaaacggacagccagagaataattataagacaactcctcccgttctggattctgacggcagcttctttctgtactctaggcttactgtggacaaaagtcgctggcaagaagggaacgtcttttcatgttctgttatgcacgaggccttgcacaatcattatacacagaagtctctgagtctctcactgggcaaaggcgggggaggcagcgggggaggcgggtccggaggcgggggatctcatcccatccctgactccagtcctctcctgcaattcgggggccaagtccggcagcggtacctctacacagatgatgctcagcagacagaagcccacctggagatcagggaggatgggaccgtggggggcgctgctgaccagagccccgaaagtctcctgcagctgaaagccttgaagcctggagttattcaaatcttgggagtcaagactagtaggttcctgtgccagcggccagatggggccctgtatggatctctccattttgaccctgaggcctgcagcttccgggagctgcttcttgaggacggatacaatgtttaccagtccgaagcccacggcctccctctgcatctgcccgggaacaagtctcctcaccgggaccctgcccccagaggacctgctcgcttcctgccactcccaggcctgccccccgcattgcctgagccacccggaatcctggccccccagccccctgatgtgggatcctctgaccctctgagcatggtgaacccttcccagggcagaagccccagctacgcttcc

SEQ ID NO: 50 - DNA, 1257 bp, Artificial Sequence
  nucleic acid molecule coding for DFD6_E-coli
gagaccaaaaccccggaatgcccttcgcatacgcagcctttgggtgtctttctctttccaccaaagccgaaagatacgcttatgatctctcgtacgccagaagttacctgcgtagtggtcgatgtttcacaggaagatcccgaagtacagtttaattggtacgtagacggtgtagaagtccataatgctaaaacaaaaccgagagaagaacagtttaattcaacgtatcgggtggttagcgttctgaccgttctgcatcaagattggctgaacgggaaagaatataaatgcaaagtaagcaataaagggctgccaagctctatcgaaaagactatatccaaggcaaaaggacaaccacgtgagccgcaagtttacacattgcctccatctcaggaggaaatgacaaaaaatcaggtttcgttaacctgtcttgttaagggtttttatcctagtgatattgcagttgaatgggaatcaaatggtcagccggaaaacaattataaaactactccgcctgttctagattctgacggttcattcttcttgtattcgcggctcactgttgataaatctcgttggcaggagggtaatgtattcagctgtagcgttatgcacgaagcactgcacaaccattacacccagaaaagcttgagcttaagcctgggtaaaggtggtggtggtagtggtggaggaggttcaggtggtggtggtagccatcctatcccagatagttctccgcttctgcagtttgggggtcaagtgcgacaacgttatctgtatactgatgatgcacagcaaaccgaagcacatcttgaaattcgtgaagacggtacagttggaggtgcagcagatcaatccccggagtcgctgttacagttgaaagcgctgaaaccgggtgttatacagattctgggtgttaaaacatcacgttttctttgtcagcgtcccgatggggctttatatgggtctctgcatttcgacccagaagcttgttcttttcgtgaactgcttctggaagacggctataatgtttatcaaagtgaagcacatggtctgccattacatctgccgggtaacaaatcaccacaccgtgatcctgcaccgagaggtccagctcgttttttacctctgcccggtctacccccggcattacccgaaccacctgggattctggcaccgcaaccgcctgatgttggaagcagtgatccgttaagtatggttaacccgagtcagggtaggagccccagctatgcgtca

SEQ ID NO: 51 - DNA, 1257 bp, Artificial Sequence
  nucleic acid molecule coding for DFD7
gagaccaagacacctgaatgtccaagtcacactcagcctctgggagtgtttctcttcccacctaagcccaaggatacccttatgatttctaggacacctgaggtgacctgcgtcgttgtggacgtgagtcaagaggacccagaggtccagtttaactggtatgttgacggcgtggaagtgcataatgcaaaaactaaaccccgcgaggaacaattcaattcaacctaccgggtcgtttctgtgttgacagtgctgcatcaagattggctgaacgggaaggagtataagtgtaaagtcagtaataagggactcccctctagtatcgaaaaaactatttcaaaggccaaaggccagcctagagagccacaggtgtacacccttcctccatcccaagaggagatgacaaagaaccaggtgtctctgacttgtctcgtgaaggggttctaccctagtgacatcgctgtcgaatgggagtcaaacggacagccagagaataattataagacaactcctcccgttctggattctgacggcagcttctttctgtactctaggcttactgtggacaaaagtcgctggcaagaagggaacgtcttttcatgttctgttatgcacgaggccttgcacaatcattatacacagaagtctctgagtctctcactgggcaaaggcgggggaggcagcgggggaggcgggtccggaggcgggggatctcatcccatccctgactccagtcctctcctgcaattcgggggccaagtccggcagcggtacctctacacagatgatgctcagcagacagaagcccacctggagatcagggaggatgggaccgtggggggcgctgctgaccagagccccgaaagtctcctgcagctgaaagccttgaagcctggagttattcaaatcttgggagtcaagactagtaggttcctgtgccagcggccagatggggccctgtatggatctctccattttgaccctgaggcctgcagcttccgggagctgcttcttgaggacggatacaatgtttaccagtccgaagcccacggcctccctctgcatctgcccgggaacaagtctcctcaccgggaccctgcccccagaggacctgctcgcttcctgccactcccaggcctgccccccgcattgcctgagccacccggaatcctggccccccagccccctgatgtgggatcctctgaccctctgagcatggtgggaccttcccagaacagaagccccagctacgcttcc

SEQ ID NO: 52 - DNA, 1257 bp, Artificial Sequence
  nucleic acid molecule coding for DFD9
gagaccaagacacctgaatgtccaagtcacactcagcctctgggagtgtttctcttcccacctaagcccaaggatacccttatgatttctaggacacctgaggtgacctgcgtcgttgtggacgtgagtcaagaggacccagaggtccagtttaactggtatgttgacggcgtggaagtgcataatgcaaaaactaaaccccgcgaggaacaattcaattcaacctaccgggtcgtttctgtgttgacagtgctgcatcaagattggctgaacgggaaggagtataagtgtaaagtcagtaataagggactcccctctagtatcgaaaaaactatttcaaaggccaaaggccagcctagagagccacaggtgtacacccttcctccatcccaagaggagatgacaaagaaccaggtgtctctgacttgtctcgtgaaggggttctaccctagtgacatcgctgtcgaatgggagtcaaacggacagccagagaataattataagacaactcctcccgttctggattctgacggcagcttctttctgtactctaggcttactgtggacaaaagtcgctggcaagaagggaacgtcttttcatgttctgttatgcacgaggccttgcacaatcattatacacagaagtctctgagtctctcactgggcaaaggcgggggaggcagcgggggaggcgggtccggaggcgggggatctcatcccatccctgactccagtcctctcctgcaattcgggggccaagtccggcagcggtacctctacacagatgatgctcagcagacagaagcccacctggagatcagggaggatgggaccgtggggggcgctgctgaccagagccccgaaagtctcctgcagctgaaagccttgaagcctggagttattcaaatcttgggagtcaagactagtaggttcctgtgccagcggccagatggggccctgtatggatctctccattttgaccctgaggcctgcagcttccgggagctgcttcttgaggacggatacaatgtttaccagtccgaagcccacggcctccctctgcatctgcccgggaacaagtctcctcaccgggaccctgcccccagaggacctgctcgcttcctgccactcccaggcctgccccccgcattgcctgagccacccggaatcctggccccccagccccctgatgtgggatcctctgaccctctgagcatggtgggaccttcccagggcagaagccccagctacgcttcc

SEQ ID NO: 53 - DNA, 1260 bp, Artificial Sequence
  nucleic acid molecule coding for DFD13
gagaccaagacacctgaatgtccaagtcacactcagcctctgggagtgtttctcttcccacctaagcccaaggatacccttatgatttctaggacacctgaggtgacctgcgtcgttgtggacgtgagtcaagaggacccagaggtccagtttaactggtatgttgacggcgtggaagtgcataatgcaaaaactaaaccccgcgaggaacaattcaattcaacctaccgggtcgtttctgtgttgacagtgctgcatcaagattggctgaacgggaaggagtataagtgtaaagtcagtaataagggactcccctctagtatcgaaaaaactatttcaaaggccaaaggccagcctagagagccacaggtgtacacccttcctccatcccaagaggagatgacaaagaaccaggtgtctctgacttgtctcgtgaaggggttctaccctagtgacatcgctgtcgaatgggagtcaaacggacagccagagaataattataagacaactcctcccgttctggattctgacggcagcttctttctgtactctaggcttactgtggacaaaagtcgctggcaagaagggaacgtcttttcatgttctgttatgcacgaggccttgcacaatcattatacacagaagtctctgagtctctcactgggcaaaggcgggggaggcagcgggggaggcgggtccggaggcgggggatctcatcccatccctgactccagtcctctcctgcaattcgggggccaagtccggcagcggtacctctacacagatgatgctcagcagacagaagcccacctggagatcagggaggatgggaccgtggggggcgctgctgaccagagccccgaaagtctcctgcagctgaaagccttgaagcctggagttattcaaatcttgggagtcaagactagtaggttcctgtgccagcggccagatggggccctgtatggatctctccattttgaccctgaggcctgcagcttccgggaggagatcagacccgacggatacaatgtttaccagtccgaagcccacggcctccctctgcatctgcccgggaacaagtctcctcaccgggaccctgcccccagaggacctgctcgcttcctgccactcccaggcctgccccccgcattgcctgagccacccggaatcctggccccccagccccctgatgtgggatcctctgaccctctgagcatggtgacaggcctggaggccgtgagaagccccagctacgcttcc

SEQ ID NO: 54 - DNA, 1260 bp, Artificial Sequence
  nucleic acid molecule coding for DFD18
gagaccaagacacctgaatgtccaagtcacactcagcctctgggagtgtttctcttcccacctaagcccaaggatacccttatgatttctaggacacctgaggtgacctgcgtcgttgtggacgtgagtcaagaggacccagaggtccagtttaactggtatgttgacggcgtggaagtgcataatgcaaaaactaaaccccgcgaggaacaattcaattcaacctaccgggtcgtttctgtgttgacagtgctgcatcaagattggctgaacgggaaggagtataagtgtaaagtcagtaataagggactcccctctagtatcgaaaaaactatttcaaaggccaaaggccagcctagagagccacaggtgtacacccttcctccatcccaagaggagatgacaaagaaccaggtgtctctgacttgtctcgtgaaggggttctaccctagtgacatcgctgtcgaatgggagtcaaacggacagccagagaataattataagacaactcctcccgttctggattctgacggcagcttctttctgtactctaggcttactgtggacaaaagtcgctggcaagaagggaacgtcttttcatgttctgttatgcacgaggccttgcacaatcattatacacagaagtctctgagtctctcactgggcaaaggcgggggaggcagcgggggaggcgggtccggaggcgggggatctcatcccatccctgactccagtcctctcctgcaattcgggggccaagtccggcagcggtacctctacacagatgatgctcagcagacagaagcccacctggagatcagggaggatgggaccgtggggggcgctgctgaccagagccccgaaagtctcctgcagctgaaagccttgaagcctggagttattcaaatcttgggagtcaagactagtaggttcctgtgccagcggccagatggggccctgtatggatctctccattttgaccctgaggcctgcagcttccgggaggagatcagacccgacggatacaatgtttaccagtccgaagcccacggcctccctctgcatctgcccgggaacaagtctcctcaccgggaccctgcccccagaggacctgctcgcttcctgccactcccaggcctgccccccgcattgcctgagccacccggaatcctggccccccagccccctgatgtgggatcctctgaccctctgagcatggtgacaggcctggaggccgtgagaagccccagctacgagtcc

SEQ ID NO: 55 - DNA, 1260 bp, Artificial Sequence
  nucleic acid molecule coding for DFD72
gagaccaagacacctgaatgtccaagtcacactcagcctctgggagtgtttctcttcccacctaagcccaaggatacccttatgatttctaggacacctgaggtgacctgcgtcgttgtggacgtgagtcaagaggacccagaggtccagtttaactggtatgttgacggcgtggaagtgcataatgcaaaaactaaaccccgcgaggaacaattcaattcaacctaccgggtcgtttctgtgttgacagtgctgcatcaagattggctgaacgggaaggagtataagtgtaaagtcagtaataagggactcccctctagtatcgaaaaaactatttcaaaggccaaaggccagcctagagagccacaggtgtacacccttcctccatcccaagaggagatgacaaagaaccaggtgtctctgacttgtctcgtgaaggggttctaccctagtgacatcgctgtcgaatgggagtcaaacggacagccagagaataattataagacaactcctcccgttctggattctgacggcagcttctttctgtactctaggcttactgtggacaaaagtcgctggcaagaagggaacgtcttttcatgttctgttatgcacgaggccttgcacaatcattatacacagaagtctctgagtctctcactgggcaaaggcgggggaggcagcgggggaggcgggtccggaggcgggggatctcatcccatccctgactccagtcctctcctgcaattcgggggccaagtccggcagcggtacctctacacagatgatgctcagcagacagaagcccacctggagatcagggaggatgggaccgtggggggcgctgctgaccagagccccgaaagtctcctgcagctgaaagccttgaagcctggagttattcaaatcttgggagtcaagactagtaggttcctgtgccagcggccagatggggccctgtatggatctctccattttgaccctgaggcctgcagcttccgggaggagatcagacccgacggatacaatgtttaccagtccgaagcccacggcctccctctgcatctgcccgggaacaagtctcctcaccgggaccctgcccccagaggacctgctcgcttcctgccactcccaggcctgccccccgcattgcctgagccacccggaatcctggccccccagccccctgatgtgggatcctctgaccctctgagcatggtgacaggcctggaggccaacagaagccccagctacgagtcc

SEQ ID NO: 56 - DNA, 1257 bp, Artificial Sequence
  nucleic acid molecule coding for DFD73
gagaccaagacacctgaatgtccaagtcacactcagcctctgggagtgtttctcttcccacctaagcccaaggatacccttatgatttctaggacacctgaggtgacctgcgtcgttgtggacgtgagtcaagaggacccagaggtccagtttaactggtatgttgacggcgtggaagtgcataatgcaaaaactaaaccccgcgaggaacaattcaattcaacctaccgggtcgtttctgtgttgacagtgctgcatcaagattggctgaacgggaaggagtataagtgtaaagtcagtaataagggactcccctctagtatcgaaaaaactatttcaaaggccaaaggccagcctagagagccacaggtgtacacccttcctccatcccaagaggagatgacaaagaaccaggtgtctctgacttgtctcgtgaaggggttctaccctagtgacatcgctgtcgaatgggagtcaaacggacagccagagaataattataagacaactcctcccgttctggattctgacggcagcttctttctgtactctaggcttactgtggacaaaagtcgctggcaagaagggaacgtcttttcatgttctgttatgcacgaggccttgcacaatcattatacacagaagtctctgagtctctcactgggcaaaggcgggggaggcagcgggggaggcgggtccggaggcgggggatctcatcccatccctgactccagtcctctcctgcaattcgggggccaagtccggcagcggtacctctacacagatgatgctcagcagacagaagcccacctggagatcagggaggatgggaccgtggggggcgctgctgaccagagccccgaaagtctcctgcagctgaaagccttgaagcctggagttattcaaatcttgggagtcaagactagtaggttcctgtgccagcggccagatggggccctgtatggatctctccattttgaccctgaggcctgcagcttccgggaggagatcagacccgacggatacaatgtttaccagtccgaagcccacggcctccctctgcatctgcccgggaacaagtctcctcaccgggaccctgcccccagaggacctgctcgcttcctgccactcccaggcctgccccccgcattgcctgagccacccggaatcctggccccccagccccctgatgtgggatcctctgaccctctgagcatggtgaacccttcccagggcagaagccccagctacgcttcc

SEQ ID NO: 57 - DNA, 1257 bp, Artificial Sequence
  nucleic acid molecule coding for DFD74
gagaccaagacacctgaatgtccaagtcacactcagcctctgggagtgtttctcttcccacctaagcccaaggatacccttatgatttctaggacacctgaggtgacctgcgtcgttgtggacgtgagtcaagaggacccagaggtccagtttaactggtatgttgacggcgtggaagtgcataatgcaaaaactaaaccccgcgaggaacaattcaattcaacctaccgggtcgtttctgtgttgacagtgctgcatcaagattggctgaacgggaaggagtataagtgtaaagtcagtaataagggactcccctctagtatcgaaaaaactatttcaaaggccaaaggccagcctagagagccacaggtgtacacccttcctccatcccaagaggagatgacaaagaaccaggtgtctctgacttgtctcgtgaaggggttctaccctagtgacatcgctgtcgaatgggagtcaaacggacagccagagaataattataagacaactcctcccgttctggattctgacggcagcttctttctgtactctaggcttactgtggacaaaagtcgctggcaagaagggaacgtcttttcatgttctgttatgcacgaggccttgcacaatcattatacacagaagtctctgagtctctcactgggcaaaggcgggggaggcagcgggggaggcgggtccggaggcgggggatctcatcccatccctgactccagtcctctcctgcaattcgggggccaagtccggcagcggtacctctacacagatgatgctcagcagacagaagcccacctggagatcagggaggatgggaccgtggggggcgctgctgaccagagccccgaaagtctcctgcagctgaaagccttgaagcctggagttattcaaatcttgggagtcaagactagtaggttcctgtgccagcggccagatggggccctgtatggatctctccattttgaccctgaggcctgcagcttccgggaggagatcagacccgacggatacaatgtttaccagtccgaagcccacggcctccctctgcatctgcccgggaacaagtctcctcaccgggaccctgcccccagaggacctgctcgcttcctgccactcccaggcctgccccccgcattgcctgagccacccggaatcctggccccccagccccctgatgtgggatcctctgaccctctgagcatggtgaacccttcccagggcagaagccccagctacgagtcc

SEQ ID NO: 58 - protein, 25 aa, Artificial Sequence
  leader sequence
MDAMLRGLCCVLLLCGAVFVSPSHA